European Patent Specification EP 3 500 595 B1, published May 1, 2024. Title: Antibodies, uses thereof and conjugates thereof. Applicant: Polytherics Limited. The sequence listing filed with the application follows.

SEQUENCE LISTING (38 sequences)

SEQ ID NO: 1 - protein, 115 aa, synthetic construct
EVQLQQSGPELKKPGTSVRISCKTSGYTFTEYTIHWVKQSHGKSLEWIGNINPNNGGTTYNQKFEDKATLTVDKSSSTAYMELRSLTSEDSAVYYCAAGWNFDYWGQGTTLTVSS

SEQ ID NO: 2 - protein, 107 aa, synthetic construct
DIVMTQSHKFMSTSVGDRVSIICKASQDVGTAVDWYQQKPGQSPKLLIYWASTRHTGVPDRFTGSGSGTDFTLTITNVQSEDLADYFCQQYNSYPLTFGAGTMLDLK

SEQ ID NO: 3 - protein, 115 aa, synthetic construct
EVQLVQSGPEVKKPGATVKISCKTSGYTFTEYTIHWVKQAPGKGLEWIGNINPNNGGTTYNQKFEDKATLTVDKSTDTAYMELSSLRSEDTAVYYCAAGWNFDYWGQGTLLTVSS

SEQ ID NO: 4 - protein, 107 aa, synthetic construct
DIQMTQSPSSLSTSVGDRVTLTCKASQDVGTAVDWYQQKPGPSPKLLIYWASTRHTGIPSRFSGSGSGTDFTLTISSLQPEDFADYYCQQYNSYPLTFGPGTKVDIK

SEQ ID NO: 5 - protein, 115 aa, synthetic construct
EVQLVQSGAEVKKPGASVKVSCKASGYTFTEYTIHWVRQAPGKGLEWIGNINPNNGGTTYNQKFEDRVTITVDKSTSTAYMELSSLRSEDTAVYYCAAYWLFDYWGQGTTVTVSS

SEQ ID NO: 6 - protein, 107 aa, synthetic construct
DIQMTQSPSTLSASVGDRVTITCKASQDVGTAVDWYQQKPGQAPKLLIYWASTRHTGVPDRFSGSGSGTDFTLTISRLQPEDFAVYYCQQYNSYPLTFGQGTKVDIK

SEQ ID NO: 7 - protein, 115 aa, synthetic construct
EVQLVQSGAEVKKPGASVKVSCKASGYTFTEYTIHWVRQAPGKGLEWIGNINPNNGGTTYNQKFEDRVTITVDKSTSTAYMELSSLRSEDTAVYYCAGGWTFDYWGQGTTVTVSS

SEQ ID NO: 8 - protein, 107 aa, synthetic construct
DIQMTQSPSTLSASVGDRVTITCKASQDVGTAVDWYQQKPGQAPKLLIYWASTRHTGVPDRFSGSGSGTDFTLTISRLQPEDFAVYYCQQFTRYPLTFGQGTKVDIK

SEQ ID NO: 9 - protein, 115 aa, synthetic construct
EVQLVQSGAEVKKPGASVKVSCKASGYTFTEYTIHWVRQAPGKGLEWIGNINPNNGGTTYNQKFEDRVTITVDKSTSTAYMELSSLRSEDTAVYYCAGAWTMDYWGQGTTVTVSS

SEQ ID NO: 10 - protein, 107 aa, synthetic construct
DIQMTQSPSTLSASVGDRVTITCKASQDVGTAVDWYQQKPGQAPKLLIYWASTRHTGVPDRFSGSGSGTDFTLTISRLQPEDFAVYYCQQYNAYSLTFGQGTKVDIK

SEQ ID NO: 11 - protein, 115 aa, synthetic construct
EVQLVQSGAEVKKPGASVKVSCKASGYTFTEYTIHWVRQAPGKGLEWIGNINPNNGGTTYNQKFEDRVTITVDKSTSTAYMELSSPRSEDTAVYYCAAGWNFDYWGQGTTVTVSS

SEQ ID NO: 12 - protein, 115 aa, synthetic construct
EVQLVQSGAEVKKPGASVKVSCKASGYTFTEYTIHWVRQAPGKGLEWIGNINPNNGGTTYNQKFEDRVTITVDKSTSTAYMELSSLRSEDTAVYYCAAGWNFDYWGQGTTVTVSS

SEQ ID NO: 13 - protein, 142 aa, synthetic construct
MELGLRWGFLVALLRGVQCQVQLVESGGGVVQPGRSLRLSCAASGFAFSRYGMHWVRQAPGKGLEWVAVIWYDGSNKYYADSVKGRFTISRDNSKNTQYLQMNSLRAEDTAVYYCARGGDFLYYYYYGMDVWGQGTTVTVSS

SEQ ID NO: 14 - protein, 127 aa, synthetic construct
MRVPAQLLGLLLLWLPDTRCDIQMTQSPSSLSASVGDRVTITCRASQGISNYLAWYQQKTGKVPKFLIYEASTLQSGVPSRFSGGGSGTDFTLTISSLQPEDVATYYCQNYNSAPFTFGPGTKVDIK

SEQ ID NO: 15 - protein, 143 aa, synthetic construct
MELGLRWVLLVALLRGVQCQVQLVESGGGVVQPGRSLRLSCAASGFTFSNYVMHWVRQAPGKGLEWVAIIWYDGSNKYYADSVKGRFTISRDNSKNTLYLQMNSLRAEDTAVYYCAGGYNWNYEYHYYGMDVWGQGTTVTVSS

SEQ ID NO: 16 - protein, 127 aa, synthetic construct
MRVPAQLLGLLLLCFPGARCDIQMTQSPSSLSASVGDRVTITCRASQGITNYLAWFQQKPGKAPKSLIYAASSLQSGVPSKFSGSGSGTDFSLTISSLQPEDFATYYCQQYNSYPITFGQGTRLEIK

SEQ ID NO: 17 - DNA, 345 bp, synthetic construct
gaggtccagctgcaacagtctggacctgagctgaagaagcctgggacttcagtgaggatatcctgcaagacttctggatacacattcactgaatacaccatccactgggtgaagcagagccatggaaagagccttgagtggattggaaacattaatcctaacaatggtggtactacctacaaccagaagttcgaggacaaggccacattgactgtagacaagtcctccagcacagcctacatggagctccgcagcctgacatctgaggattctgcagtctattactgtgcagctggttggaactttgactactggggccaaggcaccacgctcaccgtctcctca

SEQ ID NO: 18 - DNA, 321 bp, synthetic construct
gacattgtgatgacccagtctcacaaattcatgtccacatcagtaggagacagggtcagcatcatctgcaaggccagtcaggatgtgggtactgctgtagactggtatcaacagaaaccagggcaatctcctaaactactgatttactgggcatccacccggcacactggagtccctgatcgcttcacaggcagtggatctgggacagatttcactctcaccatcaccaatgtgcagtctgaagacctggcagattatttctgtcagcaatataacagctatcctctcacgttcggcgccgggaccatgctggatctcaaa

SEQ ID NO: 19 - DNA, 345 bp, synthetic construct
gaggtccaactggtacagtctggacctgaagtgaagaagcctggggctacagtgaagatatcctgcaagacttctggatacacattcactgaatataccatacactgggtgaagcaggcccctggaaagggccttgagtggattggaaacatcaatcctaacaatggtggtaccacctacaatcagaagttcgaggacaaggccacactaactgtagacaagtccaccgatacagcctacatggagctcagcagcctaagatctgaggatactgcagtctattattgtgcagctggttggaactttgactactggggccaagggaccctgctcaccgtctcctca

SEQ ID NO: 20 - DNA, 321 bp, synthetic construct
gacatccagatgacccagtctccctcatccctgtccacatcagtaggagacagggtcaccctcacctgtaaggccagtcaagatgtgggtactgctgtagactggtatcaacagaaaccaggaccatctcctaaactactgatttattgggcatccactcggcacactggaatccctagtcgcttctcaggcagtggatctgggacagacttcactctcaccatttctagtcttcagcctgaagactttgcagattattactgtcagcaatataacagctatcctctcacgttcggtcctgggaccaaggtggacatcaaa

SEQ ID NO: 21 - DNA, 345 bp, synthetic construct
gaggtccagctggtgcagtctggagctgaggtgaagaagcctggggcctcagtgaaggtctcctgcaaggcttctggatacacattcactgaatacaccatccactgggtgaggcaggcccctggaaagggccttgagtggattggaaacattaatcctaacaatggtggtactacctacaaccagaagttcgaggacagagtcacaatcactgtagacaagtccaccagcacagcctacatggagctcagcagcctgagatctgaggatactgcagtctattactgtgcagcttactggctgttcgactactggggccaaggcaccacggtcaccgtctcctca

SEQ ID NO: 22 - DNA, 321 bp, synthetic construct
gacattcagatgacccagtctcccagcaccctgtccgcatcagtaggagacagggtcaccatcacttgcaaggccagtcaggatgtgggtactgctgtagactggtatcaacagaaaccagggcaagctcctaaactactgatttactgggcatccacccggcacactggagtccctgatcgcttcagcggcagtggatctgggacagatttcactctcaccatcagcagactgcagcctgaagactttgcagtttattactgtcagcaatataacagctatcctctcacgttcggccaggggaccaaggtggatatcaaa

SEQ ID NO: 23 - DNA, 345 bp, synthetic construct
gaggtccagctggtgcagtctggagctgaggtgaagaagcctggggcctcagtgaaggtctcctgcaaggcttctggatacacattcactgaatacaccatccactgggtgaggcaggcccctggaaagggccttgagtggattggaaacattaatcctaacaatggtggtactacctacaaccagaagttcgaggacagagtcacaatcactgtagacaagtccaccagcacagcctacatggagctcagcagcctgagatctgaggatactgcagtctattactgtgcaggtgggtggaccttcgactactggggccaaggcaccacggtcaccgtctcctca

SEQ ID NO: 24 - DNA, 321 bp, synthetic construct
gacattcagatgacccagtctcccagcaccctgtccgcatcagtaggagacagggtcaccatcacttgcaaggccagtcaggatgtgggtactgctgtagactggtatcaacagaaaccagggcaagctcctaaactactgatttactgggcatccacccggcacactggagtccctgatcgcttcagcggcagtggatctgggacagatttcactctcaccatcagcagactgcagcctgaagactttgcagtttattactgtcagcagttcaccaggtatcctctcacgttcggccaggggaccaaggtggatatcaaa

SEQ ID NO: 25 - DNA, 345 bp, synthetic construct
gaggtccagctggtgcagtctggagctgaggtgaagaagcctggggcctcagtgaaggtctcctgcaaggcttctggatacacattcactgaatacaccatccactgggtgaggcaggcccctggaaagggccttgagtggattggaaacattaatcctaacaatggtggtactacctacaaccagaagttcgaggacagagtcacaatcactgtagacaagtccaccagcacagcctacatggagctcagcagcctgagatctgaggatactgcagtctattactgtgcaggtgcgtggaccatggactactggggccaaggcaccacggtcaccgtctcctca

SEQ ID NO: 26 - DNA, 321 bp, synthetic construct
gacattcagatgacccagtctcccagcaccctgtccgcatcagtaggagacagggtcaccatcacttgcaaggccagtcaggatgtgggtactgctgtagactggtatcaacagaaaccagggcaagctcctaaactactgatttactgggcatccacccggcacactggagtccctgatcgcttcagcggcagtggatctgggacagatttcactctcaccatcagcagactgcagcctgaagactttgcagtttattactgtcagcaatataacgcgtactcgttgacgttcggccaggggaccaaggtggatatcaaa

SEQ ID NO: 27 - DNA, 345 bp, synthetic construct
gaggtccagctggtgcagtctggagctgaggtgaagaagcctggggcctcagtgaaggtctcctgcaaggcttctggatacacattcactgaatacaccatccactgggtgaggcaggcccctggaaagggccttgagtggattggaaacattaatcctaacaatggtggtactacctacaaccagaagttcgaggacagagtcacaatcactgtagacaagtccaccagcacagcctacatggagctcagcagcccgagatctgaggatactgcagtctattactgtgcagctggttggaactttgactactggggccaaggcaccacggtcaccgtctcctca

SEQ ID NO: 28 - DNA, 345 bp, synthetic construct
gaggtccagctggtgcagtctggagctgaggtgaagaagcctggggcctcagtgaaggtctcctgcaaggcttctggatacacattcactgaatacaccatccactgggtgaggcaggcccctggaaagggccttgagtggattggaaacattaatcctaacaatggtggtactacctacaaccagaagttcgaggacagagtcacaatcactgtagacaagtccaccagcacagcctacatggagctcagcagcctgagatctgaggatactgcagtctattactgtgcagctggttggaactttgactactggggccaaggcaccacggtcaccgtctcctca

SEQ ID NO: 29 - protein, 115 aa, synthetic construct; identical to SEQ ID NO: 5
  varient (98)..(102): Residues as these positions are selected from the following sequences: Ala Tyr Trp Leu Phe, Gly Gly Trp Thr Phe, or Gly Ala Trp Thr Met

SEQ ID NO: 30 - protein, 115 aa, synthetic construct; identical to SEQ ID NO: 5
  varient (9)..(9): This residue is selected from Ala or Pro
  varient (11)..(11): This residue is selected from Val or Leu
  varient (24)..(24): This residue is selected from Ala or Thr
  varient (38)..(38): This residue is selected from Arg or Lys
  varient (41)..(41): This residue is selected from Pro or His
  varient (55)..(55): This residue is selected from Asn or Gln
  varient (68)..(68): This residue is selected from Val or Ala
  varient (70)..(70): This residue is selected from Ile or Leu
  varient (86)..(86): This residue is selected from Leu or Pro
  varient (98)..(102): Residues as these positions are selected from the following sequences: Ala Tyr Trp Leu Phe, Gly Gly Trp Thr Phe, or Gly Ala Trp Thr Met

SEQ ID NO: 31 - protein, 107 aa, synthetic construct; identical to SEQ ID NO: 8
  varient (91)..(95): Residues as these positions are selected from the following sequences: Phe Thr Arg Tyr Pro or Tyr Asn Ala Tyr Ser

SEQ ID NO: 32 - protein, 107 aa, synthetic construct; identical to SEQ ID NO: 8
  varient (3)..(3): This residue is selected from Gln or Val
  varient (10)..(10): This residue is selected from Thr or Phe
  varient (63)..(63): This residue is selected from Ser or Thr
  varient (80)..(80): This residue is selected from Pro or Ser
  varient (85)..(85): This residue is selected from Val or Asp
  varient (87)..(87): This residue is selected from Tyr or Phe
  varient (91)..(95): Residues as these positions are selected from the following sequences: Phe Thr Arg Tyr Pro or Tyr Asn Ala Tyr Ser
  varient (103)..(103): This residue is selected from Lys or Met

SEQ ID NO: 33 - protein, 5 aa, synthetic construct
EYTIH

SEQ ID NO: 34 - protein, 17 aa, synthetic construct
  varient (6)..(6): This residue is selected from Asn or Gln
NINPNNGGTTYNQKFED

SEQ ID NO: 35 - protein, 6 aa, synthetic construct
  varient (1)..(4): Residues as these positions are selected from the following sequences: Tyr Trp Leu Phe, Gly Trp Thr Phe or Ala Tyr Thr Met
YWLFDY

SEQ ID NO: 36 - protein, 11 aa, synthetic construct
KASQDVGTAVD

SEQ ID NO: 37 - protein, 7 aa, synthetic construct
WASTRHT

SEQ ID NO: 38 - protein, 9 aa, Artificial Sequence
  synthetic sequence
  varient (3)..(7): Residues as these positions are selected from the following sequences: Phe Thr Arg Tyr Pro or Tyr Asn Ala Tyr Ser
QQFTRYPLT